European Patent Application EP 4 365 200 A1, published May 8, 2024. Title: ANTI-CD40 ANTIBODY, ANTIGEN-BINDING FRAGMENT AND MEDICAL USE THEREOF. Applicant: JIANGSU HENGRUI PHARMACEUTICALS CO., LTD. SHANGHAI SHENGDI PHARMACEUTICAL CO., LTD. The sequence listing filed with the application follows.

SEQUENCE LISTING (100 sequences)

SEQ ID NO: 1 - protein, 114 aa, Artificial Sequence
  VH
QSVKESEGGLFKPTDTLTLTCTASRFSLSSYDMSWVRQAPGNGLEWIGAIGGAGGTYYASWAKSRSTITRNTNLNTLTLKMTSLTAADTATYFCARGWTRLDLWGQGTLVTVSS

SEQ ID NO: 2 - protein, 113 aa, Artificial Sequence
  VL
ADIVLTQTASPVSGAVGGTVTINCQSSEDISSNLSWYQQKPGQPPKLLIYAASNLASGVPSRFKGSGSGTEFTLTISDLECADAATYYCQGGYWSGISNFGNGFGGGTEVVVK

SEQ ID NO: 3 - protein, 114 aa, Artificial Sequence
  VH
QSVRESEGGLVKPTDTLTLTCTVSGFSLSSYDMSWVRQAPGNGLEWIGAIGGAGGTYYASWAKSRSTITRNTNLNTVTLKMSSLTAADTATYFCARGWTRLDLWGQGTLVTVSS

SEQ ID NO: 4 - protein, 113 aa, Artificial Sequence
  VL
ADIVLTQTPSPVSGAVGGTVTIKCQASEDISSNLAWYQQKPGQPPKLLIFPASNLASGVSSRFKGSGSGTEFTLTISDLECADAATYYCQGGYWTSTSNFGNGFGGGTEVVVK

SEQ ID NO: 5 - protein, 114 aa, Artificial Sequence
  VH
QSVKESEGGLFKPTDTLTLTCTVSGFSLSSYDMSWVRQAPGNGLEWIGAIGGAGGTYYASWAKSRSTITRNTNLNTVTLKMTSLTAADTATYFCTRGWTRLDLWGQGTLVTVSS

SEQ ID NO: 6 - protein, 113 aa, Artificial Sequence
  VL
ADIVLTQTESPVSGPVGGTVTINCQASEDISSNLAWYQQKPGQPPKLLIYAASNLASGVPSRFKGSGSGTEFTLTISDLECADAATYYCQGAYWSSTSYFGNGFGGGTQVVVK

SEQ ID NO: 7 - protein, 115 aa, Artificial Sequence
  VH
QSVKESEGGLFKPADTLTLTCTVSRFSLSSYGVTWVRQAPGNGLEWIGAIGSTGSAYYASWAKSRSTITRDTNLNTVTLKMTSLTAADTATYFCARGGITAYAIWGPGTLVTVSS

SEQ ID NO: 8 - protein, 108 aa, Artificial Sequence
  VL
AFELTQTPSSVEAAVGGTVTIKCQASQSISNGLAWYQQKPGQPPKLLIAGASNLASGVSSRFKGSGSGIEFILTISDLECADAATYYCQSYYNSFTTVFGGGTEVVVK

SEQ ID NO: 9 - protein, 115 aa, Artificial Sequence
  VH
QSVKESEGGLFKPTDTLTLTCTVSGFSLNSYGVSWVRQAPGNGLEWIGAIGSSGSAYYASWARSRSTITRDTNLNTVTLKMTSLTAADTATYFCARGGITVYAIWGPGTLVTVSS

SEQ ID NO: 10 - protein, 108 aa, Artificial Sequence
  VL
AFELTQTPSPVSAAVGGTVTINCQASEDITNGIAWYQQKPGQPPKLLIAGASNLASGVSSRFKGSGSGTEFTLTISDLECDDAATYYCQSYYSSSYTIFGGGTEVVVK

SEQ ID NO: 11 - protein, 115 aa, Artificial Sequence
  VH
QSVKESEGGLFKPTATLTLTCTVSGFSLSSYGVSWVRQAPGSGLEWIGGIASTGTTYYANWAKSRSTITRDTNLKTVTLKMTSLTAADTATYFCARGGITAYAIWGPGTLVTVSS

SEQ ID NO: 12 - protein, 108 aa, Artificial Sequence
  VL
AFELTQTPSSVEAAVGGTVTIKCQASQSITNGLAWYQQKPGQPPKLLIAGASNLASGVSSRFKGSGSGTEFTLTISDLECADAATYYCQSYYDSSSTVFGGGTEVVVK

SEQ ID NO: 13 - protein, 115 aa, Artificial Sequence
  VH
QSVKESEGGLFKPTDTLTLTCTVSGFSLSSYGVSWVRQAPGNGLEWIGGIGSDGSAYYASWAKSRATITRDTNLKTVTLEMTSLTVADTATYFCARGGITVYAIWGPGTLVTVSS

SEQ ID NO: 14 - protein, 108 aa, Artificial Sequence
  VL
AFELTQTPSPVSAAVGGTVTIKCQASQSISNGLAWYQQKPGQPPKVLIVGASNLASGVSSRFKGSGSGTEFTLSISDLECADGATYYCQSYFSSSSTVFGGGTEVVVK

SEQ ID NO: 15 - protein, 115 aa, Artificial Sequence
  VH
QSVKESEGGLFKPTDTLTLTCTVSGFSLSSYGVSWVRQAPGNGLEWIGGIGSDGSAYYASWAKSRATITRDTNLKTVTLEMTSLTAADTATYFCARGGITVYAIWGPGTLVTVSS

SEQ ID NO: 16 - protein, 108 aa, Artificial Sequence; identical to SEQ ID NO: 14
  VL

SEQ ID NO: 17 - protein, 115 aa, Artificial Sequence
  VH
QSVKESEGGLFKPKDTLTLTCTVSGFSLSSYGVSWVRQAPGNGLEWIGGIGSDGSAYYASWAKSRATITRDTNLKTVTLEMTSLTAADTATYFCARGGITVYAMWGPGTLVTVSS

SEQ ID NO: 18 - protein, 108 aa, Artificial Sequence
  VL
AFELTQTPASVEAAMGGTVTIKCQASQSISNGLAWYQQKPGQPPKLLIVGASNLASGVSSRFKGSGSGTEFTLSISDLECADGATYYCQSYFSSSSTVFGGGTEVVVK

SEQ ID NO: 19 - protein, 124 aa, Artificial Sequence
  VH
QSVKESEGGLFKPTDTLTLTCTVSGFSLSSYAISWVRQAPGNGLEWIGAIDRYGTTYYATWAKSRSTITRNTNENTVTLKMTSLTAADTATYFCARGPWYYGGDVAWTGSFDPWGPGTLVTVSS

SEQ ID NO: 20 - protein, 110 aa, Artificial Sequence
  VL
AQVLTQTASPVSAAVGGTVTISCQSSQSVANNDFLSWYQQKPGQPPKLLIYGASTLASGVPSRFRGNGSGTQFTLTITGMQCDDAATYFCTGGYAGPIYIFGGGTEVVVK

SEQ ID NO: 21 - protein, 123 aa, Artificial Sequence
  VH
QSLEESGGRLVTPGGSLTLTCTVSGIDLSRNAISWVRQSPGNGLEWIGGIGSSGSAYYASWAKSRSTITRDTNLNTVTLKMTSLTAADTATYFCARDGYAGSSWGIYYGMDPWGPGTLVTVSS

SEQ ID NO: 22 - protein, 110 aa, Artificial Sequence
  VL
AIEMTQSPPSLSASVGETVRIRCLASEDIYRGISWYQQKPGKPPTLLIYGASTLQSGVPPRFSGSGSGTDYTLTIGGVQAEDAATYYCLGGHSYSSAGLTFGAGTKVEIK

SEQ ID NO: 23 - protein, 5 aa, Artificial Sequence
  CDR
SYDMS

SEQ ID NO: 24 - protein, 16 aa, Artificial Sequence
  CDR
AIGGAGGTYYASWAKS

SEQ ID NO: 25 - protein, 7 aa, Artificial Sequence
  CDR
GWTRLDL

SEQ ID NO: 26 - protein, 11 aa, Artificial Sequence
  CDR
QSSEDISSNLS

SEQ ID NO: 27 - protein, 7 aa, Artificial Sequence
  CDR
AASNLAS

SEQ ID NO: 28 - protein, 14 aa, Artificial Sequence
  CDR
QGGYWSGISNFGNG

SEQ ID NO: 29 - protein, 11 aa, Artificial Sequence
  CDR
QASEDISSNLA

SEQ ID NO: 30 - protein, 7 aa, Artificial Sequence
  CDR
PASNLAS

SEQ ID NO: 31 - protein, 14 aa, Artificial Sequence
  CDR
QGGYWTSTSNFGNG

SEQ ID NO: 32 - protein, 14 aa, Artificial Sequence
  CDR
QGAYWSSTSYFGNG

SEQ ID NO: 33 - protein, 5 aa, Artificial Sequence
  CDR
SYGVT

SEQ ID NO: 34 - protein, 16 aa, Artificial Sequence
  CDR
AIGSTGSAYYASWAKS

SEQ ID NO: 35 - protein, 8 aa, Artificial Sequence
  CDR
GGITAYAI

SEQ ID NO: 36 - protein, 11 aa, Artificial Sequence
  CDR
QASQSISNGLA

SEQ ID NO: 37 - protein, 7 aa, Artificial Sequence
  CDR
GASNLAS

SEQ ID NO: 38 - protein, 10 aa, Artificial Sequence
  CDR
QSYYNSFTTV

SEQ ID NO: 39 - protein, 5 aa, Artificial Sequence
  CDR
SYGVS

SEQ ID NO: 40 - protein, 16 aa, Artificial Sequence
  CDR
AIGSSGSAYYASWARS

SEQ ID NO: 41 - protein, 8 aa, Artificial Sequence
  CDR
GGITVYAI

SEQ ID NO: 42 - protein, 11 aa, Artificial Sequence
  CDR
QASEDITNGIA

SEQ ID NO: 43 - protein, 10 aa, Artificial Sequence
  CDR
QSYYSSSYTI

SEQ ID NO: 44 - protein, 16 aa, Artificial Sequence
  CDR
GIASTGTTYYANWAKS

SEQ ID NO: 45 - protein, 11 aa, Artificial Sequence
  CDR
QASQSITNGLA

SEQ ID NO: 46 - protein, 10 aa, Artificial Sequence
  CDR
QSYYDSSSTV

SEQ ID NO: 47 - protein, 16 aa, Artificial Sequence
  CDR
GIGSDGSAYYASWAKS

SEQ ID NO: 48 - protein, 10 aa, Artificial Sequence
  CDR
QSYFSSSSTV

SEQ ID NO: 49 - protein, 8 aa, Artificial Sequence
  CDR
GGITVYAM

SEQ ID NO: 50 - protein, 7 aa, Artificial Sequence
  CDR
GASNLAS

SEQ ID NO: 51 - protein, 5 aa, Artificial Sequence
  CDR
SYAIS

SEQ ID NO: 52 - protein, 16 aa, Artificial Sequence
  CDR
AIDRYGTTYYATWAKS

SEQ ID NO: 53 - protein, 17 aa, Artificial Sequence
  CDR
GPWYYGGDVAWTGSFDP

SEQ ID NO: 54 - protein, 13 aa, Artificial Sequence
  CDR
QSSQSVANNDFLS

SEQ ID NO: 55 - protein, 7 aa, Artificial Sequence
  CDR
GASTLAS

SEQ ID NO: 56 - protein, 10 aa, Artificial Sequence
  CDR
TGGYAGPIYI

SEQ ID NO: 57 - protein, 5 aa, Artificial Sequence
  CDR
RNAIS

SEQ ID NO: 58 - protein, 16 aa, Artificial Sequence
  CDR
GIGSSGSAYYASWAKS

SEQ ID NO: 59 - protein, 16 aa, Artificial Sequence
  CDR
DGYAGSSWGIYYGMDP

SEQ ID NO: 60 - protein, 11 aa, Artificial Sequence
  CDR
LASEDIYRGIS

SEQ ID NO: 61 - protein, 7 aa, Artificial Sequence
  CDR
GASTLQS

SEQ ID NO: 62 - protein, 12 aa, Artificial Sequence
  CDR
LGGHSYSSAGLT

SEQ ID NO: 63 - protein, 112 aa, Artificial Sequence
  9E6-L1
DIQLTQSPSFLSASVGDRVTITCQASEDISSNLAWYQQKPGKPPKLLIFPASNLASGVPSRFSGSGSGTEFTLTISSLQPEDFATYYCQGGYWTSTSNFGNVFGGGTKVEIK

SEQ ID NO: 64 - protein, 112 aa, Artificial Sequence
  9E6-L2
DIQLTQSPSFLSASVGDRVTITCQASEDISSNLAWYQQKPGKPPKLLIFPASNLASGVPSRFSGSGSGTEFTLTISSLQPEDFATYYCQGGYWTSTSNFGSGFGGGTKVEIK

SEQ ID NO: 65 - protein, 112 aa, Artificial Sequence
  9E6-L3
DIQLTQSPSFLSASVGDRVTITCQASEDISSNLAWYQQKPGKPPKLLIFPASNLASGVPSRFSGSGSGTEFTLTISSLQPEDFATYYCQGGYWTSTSNFGTGFGGGTKVEIK

SEQ ID NO: 66 - protein, 112 aa, Artificial Sequence
  9E6-L4
DIQLTQSPSFLSASVGDRVTITCQASEDISSNLAWYQQKPGKPPKLLIFPASNLASGVPSRFSGSGSGTEFTLTISSLQPEDFATYYCQGGYWTSTSNFGQGFGGGTKVEIK

SEQ ID NO: 67 - protein, 115 aa, Artificial Sequence
  9E6-H1
EVQLQESGPGLVKPSDTLSLTCTVSGFSLSSYDMSWIRQPPGKGLEWIGAIGGAGGTYYASWAKSRVTISVDTSLNQVSLKLSSVTAADTAVYYCARGWTRLDLWGQGTLVTVSS

SEQ ID NO: 68 - protein, 115 aa, Artificial Sequence
  9E6-H2
QVQVQESGPGLVKPSDTLSLTCTVSGFSLSSYDMSWIRQPPGKGLEWIGAIGGAGGTYYASWAKSRVTISVDTSLNQVSLKLSSVTAADTAVYYCARGWTRLDLWGQGTLVTVSS

SEQ ID NO: 69 - protein, 14 aa, Artificial Sequence
  LCDR3 of 9E6-L1
QGGYWTSTSNFGNV

SEQ ID NO: 70 - protein, 14 aa, Artificial Sequence
  LCDR3 of 9E6-L2
QGGYWTSTSNFGSG

SEQ ID NO: 71 - protein, 14 aa, Artificial Sequence
  LCDR3 of 9E6-L3
QGGYWTSTSNFGTG

SEQ ID NO: 72 - protein, 14 aa, Artificial Sequence
  LCDR3 of 9E6-L4
QGGYWTSTSNFGQG

SEQ ID NO: 73 - protein, 14 aa, Artificial Sequence
  General formula for LCDR3s of 9E6-Ls
  misc_feature (13)..(14): Xaa can be any naturally occurring amino acid
QGGYWTSTSNFGXX

SEQ ID NO: 74 - protein, 11 aa, Artificial Sequence
  LCDR1
  misc_feature (2)..(2): Xaa can be any naturally occurring amino acid
  misc_feature (11)..(11): Xaa can be any naturally occurring amino acid
QXSEDISSNLX

SEQ ID NO: 75 - protein, 7 aa, Artificial Sequence
  LCDR2
  misc_feature (1)..(1): Xaa can be any naturally occurring amino acid
XASNLAS

SEQ ID NO: 76 - protein, 14 aa, Artificial Sequence
  LCDR3
  misc_feature (3)..(3): Xaa can be any naturally occurring amino acid
  misc_feature (6)..(8): Xaa can be any naturally occurring amino acid
  misc_feature (10)..(10): Xaa can be any naturally occurring amino acid
  misc_feature (13)..(14): Xaa can be any naturally occurring amino acid
QGXYWXXXSXFGXX

SEQ ID NO: 77 - protein, 108 aa, Artificial Sequence
  2F12-L1
AFQLTQSPSSLSASVGDRVTITCQASQSISNVLAWYQQKPGKPPKLLIVGASNLASGVPSRFSGSGSGTDFTLTISSLQPEDFATYYCQSYFSSSSTVFGGGTKVEIK

SEQ ID NO: 78 - protein, 108 aa, Artificial Sequence
  2F12-L2
AFQLTQSPSSLSASVGDRVTITCQASQSISQGLAWYQQKPGKPPKLLIVGASNLASGVPSRFSGSGSGTDFTLTISSLQPEDFATYYCQSYFSSSSTVFGGGTKVEIK

SEQ ID NO: 79 - protein, 108 aa, Artificial Sequence
  2F12-L3
AFQLTQSPSSLSASVGDRVTITCQASQSISSGLAWYQQKPGKPPKLLIVGASNLASGVPSRFSGSGSGTDFTLTISSLQPEDFATYYCQSYFSSSSTVFGGGTKVEIK

SEQ ID NO: 80 - protein, 108 aa, Artificial Sequence
  2F12-L4
AFQLTQSPSSLSASVGDRVTITCQASQSISTGLAWYQQKPGKPPKLLIVGASNLASGVPSRFSGSGSGTDFTLTISSLQPEDFATYYCQSYFSSSSTVFGGGTKVEIK

SEQ ID NO: 81 - protein, 116 aa, Artificial Sequence
  2F12-H1
EVTLKESGPVLVKPTETLTLTCTVSGFSLSSYGVSWIRQPPGKALEWLAGIGSDGSAYYASWAKSRLTISRDTNLKQVVLTMTNMDPVDTATYYCARGGITVYAMWGQGTLVTVSS

SEQ ID NO: 82 - protein, 116 aa, Artificial Sequence
  2F12-H2
EVTVKESGPVLVKPTETLTLTCTVSGFSLSSYGVSWIRQPPGKALEWLGGIGSDGSAYYASWAKSRLTISRDTNLKQVVLTMTNMDPVDTATYYCARGGITVYAMWGQGTLVTVSS

SEQ ID NO: 83 - protein, 11 aa, Artificial Sequence
  LCDR1 of 2F12-L1
QASQSISNVLA

SEQ ID NO: 84 - protein, 11 aa, Artificial Sequence
  LCDR1 of 2F12-L2
QASQSISQGLA

SEQ ID NO: 85 - protein, 11 aa, Artificial Sequence
  LCDR1 of 2F12-L3
QASQSISSGLA

SEQ ID NO: 86 - protein, 11 aa, Artificial Sequence
  LCDR1 of 2F12-L4
QASQSISTGLA

SEQ ID NO: 87 - protein, 11 aa, Artificial Sequence
  General formula for LCDR1s of 2F12-Ls
  misc_feature (8)..(9): Xaa can be any naturally occurring amino acid
QASQSISXXLA

SEQ ID NO: 88 - protein, 5 aa, Artificial Sequence
  HCDR1
  misc_feature (5)..(5): Xaa can be any naturally occurring amino acid
SYGVX

SEQ ID NO: 89 - protein, 16 aa, Artificial Sequence
  HCDR2
  misc_feature (1)..(1): Xaa can be any naturally occurring amino acid
  misc_feature (3)..(3): Xaa can be any naturally occurring amino acid
  misc_feature (5)..(5): Xaa can be any naturally occurring amino acid
  misc_feature (7)..(8): Xaa can be any naturally occurring amino acid
  misc_feature (12)..(12): Xaa can be any naturally occurring amino acid
  misc_feature (15)..(15): Xaa can be any naturally occurring amino acid
XIXSXGXXYYAXWAXS

SEQ ID NO: 90 - protein, 8 aa, Artificial Sequence
  HCDR3
  misc_feature (5)..(5): Xaa can be any naturally occurring amino acid
  misc_feature (8)..(8): Xaa can be any naturally occurring amino acid
GGITXYAX

SEQ ID NO: 91 - protein, 11 aa, Artificial Sequence
  LCDR1
  misc_feature (4)..(5): Xaa can be any naturally occurring amino acid
  misc_feature (7)..(9): Xaa can be any naturally occurring amino acid
QASXXIXXXLA

SEQ ID NO: 92 - protein, 10 aa, Artificial Sequence
  LCDR2
  misc_feature (4)..(5): Xaa can be any naturally occurring amino acid
  misc_feature (7)..(8): Xaa can be any naturally occurring amino acid
  misc_feature (10)..(10): Xaa can be any naturally occurring amino acid
QSYXXSXXTX

SEQ ID NO: 93 - protein, 445 aa, Artificial Sequence
  9E6-L4H2 HC
QVQVQESGPGLVKPSDTLSLTCTVSGFSLSSYDMSWIRQPPGKGLEWIGAIGGAGGTYYASWAKSRVTISVDTSLNQVSLKLSSVTAADTAVYYCARGWTRLDLWGQGTLVTVSSASTKGPSVFPLAPSSKSTSGGTAALGCLVKDYFPEPVTVSWNSGALTSGVHTFPAVLQSSGLYSLSSVVTVPSSSLGTQTYICNVNHKPSNTKVDKKVEPKSCDKTHTCPPCPAPELLGGPSVFLFPPKPKDTLMISRTPEVTCVVVDVSHEDPEVKFNWYVDGVEVHNAKTKPREEQYASTYRVVSVLTVLHQDWLNGKEYKCKVSNKALPAPIEKTISKAKGQPREPQVYTLPPSREEMTKNQVSLTCLVKGFYPSDIAVEWESNGQPENNYKTTPPVLDSDGSFFLYSKLTVDKSRWQQGNVFSCSVMHEALHNHYTQKSLSLSPGK

SEQ ID NO: 94 - protein, 219 aa, Artificial Sequence
  9E6-L4H2 LC
DIQLTQSPSFLSASVGDRVTITCQASEDISSNLAWYQQKPGKPPKLLIFPASNLASGVPSRFSGSGSGTEFTLTISSLQPEDFATYYCQGGYWTSTSNFGQGFGGGTKVEIKRTVAAPSVFIFPPSDEQLKSGTASVVCLLNNFYPREAKVQWKVDNALQSGNSQESVTEQDSKDSTYSLSSTLTLSKADYEKHKVYACEVTHQGLSSPVTKSFNRGEC

SEQ ID NO: 95 - protein, 446 aa, Artificial Sequence
  2F12-L4H2 HC
EVTVKESGPVLVKPTETLTLTCTVSGFSLSSYGVSWIRQPPGKALEWLGGIGSDGSAYYASWAKSRLTISRDTNLKQVVLTMTNMDPVDTATYYCARGGITVYAMWGQGTLVTVSSASTKGPSVFPLAPSSKSTSGGTAALGCLVKDYFPEPVTVSWNSGALTSGVHTFPAVLQSSGLYSLSSVVTVPSSSLGTQTYICNVNHKPSNTKVDKKVEPKSCDKTHTCPPCPAPELLGGPSVFLFPPKPKDTLMISRTPEVTCVVVDVSHEDPEVKFNWYVDGVEVHNAKTKPREEQYASTYRVVSVLTVLHQDWLNGKEYKCKVSNKALPAPIEKTISKAKGQPREPQVYTLPPSREEMTKNQVSLTCLVKGFYPSDIAVEWESNGQPENNYKTTPPVLDSDGSFFLYSKLTVDKSRWQQGNVFSCSVMHEALHNHYTQKSLSLSPGK

SEQ ID NO: 96 - protein, 215 aa, Artificial Sequence
  2F12-L4H2 LC
AFQLTQSPSSLSASVGDRVTITCQASQSISTGLAWYQQKPGKPPKLLIVGASNLASGVPSRFSGSGSGTDFTLTISSLQPEDFATYYCQSYFSSSSTVFGGGTKVEIKRTVAAPSVFIFPPSDEQLKSGTASVVCLLNNFYPREAKVQWKVDNALQSGNSQESVTEQDSKDSTYSLSSTLTLSKADYEKHKVYACEVTHQGLSSPVTKSFNRGEC

SEQ ID NO: 97 - protein, 445 aa, Artificial Sequence
  9E6-L4H2-AAYTE HC
QVQVQESGPGLVKPSDTLSLTCTVSGFSLSSYDMSWIRQPPGKGLEWIGAIGGAGGTYYASWAKSRVTISVDTSLNQVSLKLSSVTAADTAVYYCARGWTRLDLWGQGTLVTVSSASTKGPSVFPLAPSSKSTSGGTAALGCLVKDYFPEPVTVSWNSGALTSGVHTFPAVLQSSGLYSLSSVVTVPSSSLGTQTYICNVNHKPSNTKVDKKVEPKSCDKTHTCPPCPAPEAAGGPSVFLFPPKPKDTLYITREPEVTCVVVDVSHEDPEVKFNWYVDGVEVHNAKTKPREEQYNSTYRVVSVLTVLHQDWLNGKEYKCKVSNKALPAPIEKTISKAKGQPREPQVYTLPPSREEMTKNQVSLTCLVKGFYPSDIAVEWESNGQPENNYKTTPPVLDSDGSFFLYSKLTVDKSRWQQGNVFSCSVMHEALHNHYTQKSLSLSPGK

SEQ ID NO: 98 - protein, 446 aa, Artificial Sequence
  2F12-L4H2-AAYTE HC
EVTVKESGPVLVKPTETLTLTCTVSGFSLSSYGVSWIRQPPGKALEWLGGIGSDGSAYYASWAKSRLTISRDTNLKQVVLTMTNMDPVDTATYYCARGGITVYAMWGQGTLVTVSSASTKGPSVFPLAPSSKSTSGGTAALGCLVKDYFPEPVTVSWNSGALTSGVHTFPAVLQSSGLYSLSSVVTVPSSSLGTQTYICNVNHKPSNTKVDKKVEPKSCDKTHTCPPCPAPEAAGGPSVFLFPPKPKDTLYITREPEVTCVVVDVSHEDPEVKFNWYVDGVEVHNAKTKPREEQYNSTYRVVSVLTVLHQDWLNGKEYKCKVSNKALPAPIEKTISKAKGQPREPQVYTLPPSREEMTKNQVSLTCLVKGFYPSDIAVEWESNGQPENNYKTTPPVLDSDGSFFLYSKLTVDKSRWQQGNVFSCSVMHEALHNHYTQKSLSLSPGK

SEQ ID NO: 99 - protein, 330 aa, Artificial Sequence
  IgG1-Fc(N297A)
ASTKGPSVFPLAPSSKSTSGGTAALGCLVKDYFPEPVTVSWNSGALTSGVHTFPAVLQSSGLYSLSSVVTVPSSSLGTQTYICNVNHKPSNTKVDKKVEPKSCDKTHTCPPCPAPELLGGPSVFLFPPKPKDTLMISRTPEVTCVVVDVSHEDPEVKFNWYVDGVEVHNAKTKPREEQYASTYRVVSVLTVLHQDWLNGKEYKCKVSNKALPAPIEKTISKAKGQPREPQVYTLPPSREEMTKNQVSLTCLVKGFYPSDIAVEWESNGQPENNYKTTPPVLDSDGSFFLYSKLTVDKSRWQQGNVFSCSVMHEALHNHYTQKSLSLSPGK

SEQ ID NO: 100 - protein, 330 aa, Artificial Sequence
  IgG1-Fc(AAYTE)
ASTKGPSVFPLAPSSKSTSGGTAALGCLVKDYFPEPVTVSWNSGALTSGVHTFPAVLQSSGLYSLSSVVTVPSSSLGTQTYICNVNHKPSNTKVDKKVEPKSCDKTHTCPPCPAPEAAGGPSVFLFPPKPKDTLYITREPEVTCVVVDVSHEDPEVKFNWYVDGVEVHNAKTKPREEQYNSTYRVVSVLTVLHQDWLNGKEYKCKVSNKALPAPIEKTISKAKGQPREPQVYTLPPSREEMTKNQVSLTCLVKGFYPSDIAVEWESNGQPENNYKTTPPVLDSDGSFFLYSKLTVDKSRWQQGNVFSCSVMHEALHNHYTQKSLSLSPGK